European Patent Application EP 4 353 249 A1, published April 17, 2024. Title: MULTI AGONISTS AND APPLICATION THEREOF. Applicant: THE UNITED BIO-TECHNOLOGY (HENGQIN) CO.,LTD. The sequence listing filed with the application follows.

SEQUENCE LISTING (45 sequences)

SEQ ID NO: 1 - protein, 39 aa, Artificial Sequence
  MOD_RES (2)..(2): Xaa at position 2 is α-aminoisobutyric acid
  MOD_RES (6)..(6): Xaa at position 6 is α-methylphenylalanine
  MOD_RES (13)..(13): Xaa at position13 is α-Methylleucine
  MOD_RES (17)..(17): amino group of Lys side chain at position 7 is chemically modified by Fatty acid side chain group AEEAc-AEEAc-γGlu-CO(CH2)18COOH
  MOD_RES (20)..(20): Xaa at position 20 is Aminoisobutyric acid
  MOD_RES (38)..(38): Xaa at position 38 is Ac3c
  MOD_RES (39)..(39): Ser at position 39 is amidated optionally
YXQGTXTSDYSIXLDKKAQXAFIEYLLETGPSSGAPPXS

SEQ ID NO: 2 - protein, 39 aa, Artificial Sequence
  MOD_RES (2)..(2): Xaa at position 2 is α-aminoisobutyric acid
  MOD_RES (6)..(6): Xaa at position 6 is α-Methylphenylalanine
  MOD_RES (13)..(13): Xaa at position 13 is α-Methylleucine
  MOD_RES (17)..(17): Amino groups of Lys side chain at position 17 is chemically modified by fatty acid side chain group AEEAc-AEEAc-γGlu-CO(CH2)18COOH
  MOD_RES (20)..(20): Xaa at position 20 is α- Aminoisobutyric acid
  MOD_RES (38)..(38): Xaa at position 38 is Ac3c
  MOD_RES (39)..(39): Ser at position 39 is optionally amidated
YXQGTXTSDYSIXLDKKAQXAFIEYLLETHPSSGAPPXS

SEQ ID NO: 3 - protein, 39 aa, Artificial Sequence
  MOD_RES (2)..(2): Xaa at position 2 is α-Aminoisobutyric acid
  MOD_RES (6)..(6): Xaa at position 6 is α-Methylphenylalanine
  MOD_RES (13)..(13): Xaa at position 13 is α-Methylleucine
  MOD_RES (17)..(17): amino group of Lys side chain at position 17 is chemically modified by Fatty acid side chain group AEEAc-AEEAc-γGlu-CO(CH2)18COOH
  MOD_RES (20)..(20): Xaa at position 20 is α-Aminoisobutyric acid
  MOD_RES (38)..(38): Xaa at position 38 is Ac3c
  MOD_RES (39)..(39): Ser at position 39 is optionally amidated
YXQGTXTSDYSIXLDKKAQXAFIEYLLESHPSSGAPPXS

SEQ ID NO: 4 - protein, 39 aa, Artificial Sequence
  MOD_RES (2)..(2): Xaa at position 2 is α-Aminoisobutyric acid
  MOD_RES (6)..(6): Xaa at position 6 is α-Methyl-2-fluorophenylalanine
  MOD_RES (17)..(17): amino group of Lys side chain at position 17 is chemically modified by Fatty acid side chain groups AEEAc-AEEAc-γGlu-CO(CH2)18COOH
  MOD_RES (20)..(20): Xaa at position 20 is α-Aminoisobutyric acid
  MOD_RES (38)..(38): Xaa at position 38 is Ac3c
  MOD_RES (39)..(39): Ser at position 39 is optionally amidated
YXQGTXTSDYSIFLDKKAQXAFIEYLLEGGPSSGAPPXS

SEQ ID NO: 5 - protein, 39 aa, Artificial Sequence
  MOD_RES (2)..(2): Xaa at position 2 is α-Aminoisobutyric acid
  MOD_RES (6)..(6): Xaa at position 6 is α-Methyl-2-fluorophenylalanine
  MOD_RES (17)..(17): amino group of Lys side chain at position 17 is chemically modified by Fatty acid side chain group AEEAc-AEEAc-γGlu-CO(CH2)18COOH
  MOD_RES (20)..(20): Xaa at position 20 is α-Aminoisobutyric acid
  MOD_RES (38)..(38): Xaa at position 38 is Ac3c
  MOD_RES (39)..(39): Ser at position 39 is optionally amidated
YXQGTXTSDYSIFLDKKAQXAFIEFLLEGGPSSGAPPXS

SEQ ID NO: 6 - protein, 39 aa, Artificial Sequence
  MOD_RES (2)..(2): Xaa at position 2 is α-Aminoisobutyric acid
  MOD_RES (6)..(6): Xaa at position 6 is α-Methyl-2-fluorophenylalanine
  MOD_RES (13)..(13): Xaa at position 13 is α-Methylleucine
  MOD_RES (17)..(17): Amino group of Lys side chain at position 17 is chemically modified by Fatty acid side chain group AEEAc-AEEAc-γGlu-CO(CH2)18COOH
  MOD_RES (20)..(20): Xaa at position 20 is α-Aminoisobutyric acid
  MOD_RES (29)..(29): Xaa at position 29 is α-Aminoisobutyric acid
  MOD_RES (39)..(39): Ser at position 39 is optionally amidated
YXHGTXTSDYSIXLDKKAQXAFIEYLLEXHPSSGQPPPS

SEQ ID NO: 7 - protein, 39 aa, Artificial Sequence
  MOD_RES (2)..(2): Xaa at position 2 is α-Aminoisobutyric acid
  MOD_RES (6)..(6): Xaa at position 6 is α- Methylphenylalanine
  MOD_RES (13)..(13): Xaa at position 13 is α-Methylleucine
  MOD_RES (17)..(17): Amino group of Lys side chain at position 17 is chemically modified by Fatty acid side chain group AEEAc-AEEAc-γGlu-CO(CH2)18COOH
  MOD_RES (20)..(20): Xaa at position 20 is α-Aminoisobutyric acid
  MOD_RES (35)..(35): Xaa at position 35 is α-Aminoisobutyric acid
  MOD_RES (39)..(39): Ser at position 39 is optionally amidated
YXQGTXTSDYSIXLDKKAQXAFIEYLLETGPSSGXPPPS

SEQ ID NO: 8 - protein, 39 aa, Artificial Sequence
  MOD_RES (2)..(2): Xaa at position 2 is α- Aminoisobutyric acid
  MOD_RES (6)..(6): Xaa at position 6 is α- Methylphenylalanine
  MOD_RES (13)..(13): Xaa at position 13 is α- Methylleucine
  MOD_RES (17)..(17): Amino group of Lys side chain at position 17 is chemically modified by Fatty acid side chain group AEEAc-AEEAc-γGlu-CO(CH2)18COOH
  MOD_RES (20)..(20): Xaa at position 20 is α- Aminoisobutyric acid
  MOD_RES (39)..(39): Ser at position 39 is optionally amidated
YXQGTXTSDYSIXLDKKAQXAFIEYLLETGPSSGQPPPS

SEQ ID NO: 9 - protein, 39 aa, Artificial Sequence
  MOD_RES (2)..(2): Xaa at position 2 is α- Aminoisobutyric acid
  MOD_RES (6)..(6): Xaa at position 6 is α- Methyl-2-fluorophenylalanine
  MOD_RES (17)..(17): Amino group of Lys side chain at position 17 is chemically modified by Fatty acid side chain group AEEAc-AEEAc-γGlu-CO(CH2)18COOH
  MOD_RES (20)..(20): Xaa at position 20 is α- Aminoisobutyric acid
  MOD_RES (38)..(38): Xaa at position 38 is Ac3c
  MOD_RES (39)..(39): Ser at position 39 is optionally amidated
YXQGTXTSDYSIFLDKKAQXAFIEFLLETGPSSGAPPXS

SEQ ID NO: 10 - protein, 39 aa, Artificial Sequence
  MOD_RES (2)..(2): Xaa at position 2 is α- Aminoisobutyric acid
  MOD_RES (6)..(6): Xaa at position 6 is α- Methyl-2-fluorophenylalanine
  MOD_RES (17)..(17): Amino group of Lys side chain at position 17 is chemically modified by Fatty acid side chain group AEEAc-AEEAc-γGlu-CO(CH2)18COOH
  MOD_RES (20)..(20): Xaa at position 20 is α- Aminoisobutyric acid
  MOD_RES (38)..(38): Xaa at position 38 is Ac3c
  MOD_RES (39)..(39): Ser at position 39 is optionally amidated
YXQGTXTSDYSIFLDKKAQXAFIEFLLESHPSSGAPPXS

SEQ ID NO: 11 - protein, 39 aa, Artificial Sequence; identical to SEQ ID NO: 9
  MOD_RES (2)..(2): Xaa at position 2 is α- Aminoisobutyric acid
  MOD_RES (6)..(6): Xaa at position 6 is α- Methyl-2-fluorophenylalanine
  MOD_RES (17)..(17): Amino group of Lys side chain at position 17 is chemically modified by Fatty acid side chain group AEEAc-AEEAc-γGlu-CO(CH2)18COOH
  MOD_RES (20)..(20): Xaa at position 20 is α- Aminoisobutyric acid
  MOD_RES (38)..(38): Xaa at position 28 is Ac3c
  MOD_RES (39)..(39): Ser at position 39 is optionally amidated

SEQ ID NO: 12 - protein, 39 aa, Artificial Sequence
  MOD_RES (2)..(2): Xaa at position 2 is α- Aminoisobutyric acid
  MOD_RES (6)..(6): Xaa at position 6 is α- Methylphenylalanine
  MOD_RES (17)..(17): Amino group of Lys side chain at position 17 is chemically modified by Fatty acid side chain group AEEAc-AEEAc-γGlu-CO(CH2)18COOH
  MOD_RES (20)..(20): Xaa at position 20 is α- Aminoisobutyric acid
  MOD_RES (39)..(39): Ser at position 39 is optionally amidated
YXQGTXTSDYSIFLDKKAQXAFIEFLLETGPSSGAPPPS

SEQ ID NO: 13 - protein, 39 aa, Artificial Sequence
  MOD_RES (2)..(2): Xaa at position 2 is α- Aminoisobutyric acid
  MOD_RES (6)..(6): Xaa at position 6 is α- Methylphenylalanine
  MOD_RES (17)..(17): Amino group of Lys side chain at position 17 is chemically modified by Fatty acid side chain group AEEAc-AEEAc-γGlu-CO(CH2)18COOH
  MOD_RES (20)..(20): Xaa at position 20 is α- Aminoisobutyric acid
  MOD_RES (39)..(39): Ser at position 39 is optionally amidated
YXQGTXTSDYSIFLDKKAQXAFIEYLLETGPSSGAPPPS

SEQ ID NO: 14 - protein, 39 aa, Artificial Sequence
  MOD_RES (2)..(2): Xaa at position 2 is α- Aminoisobutyric acid
  MOD_RES (6)..(6): Xaa at position 6 is α- Methylphenylalanine
  MOD_RES (13)..(13): Xaa at position 13 is α- Methylleucine
  MOD_RES (17)..(17): Amino group of Lys side chain at position 17 is chemically modified by Fatty acid side chain group AEEAc-AEEAc-γGlu-CO(CH2)18COOH
  MOD_RES (20)..(20): Xaa at position 20 is α- Aminoisobutyric acid
  MOD_RES (39)..(39): Ser at position 39 is optionally amidated
YXQGTXTSDYSIXLDKKAQXAFIEFLLETGPSSGAPPPS

SEQ ID NO: 15 - protein, 39 aa, Artificial Sequence
  MOD_RES (2)..(2): Xaa at position 2 is α- Aminoisobutyric acid
  MOD_RES (6)..(6): Xaa at position 6 is α- Methylphenylalanine
  MOD_RES (17)..(17): Amino group of Lys side chain at position 17 is chemically modified by Fatty acid side chain group AEEAc-AEEAc-γGlu-CO(CH2)18COOH
  MOD_RES (20)..(20): Xaa at position 20 is α- Aminoisobutyric acid
  MOD_RES (39)..(39): Ser at position 39 is optionally amidated
YXQGTXTSDYSIFLDKKAQXAFIEFLLESHPSSGAPPPS

SEQ ID NO: 16 - protein, 39 aa, Artificial Sequence
  MOD_RES (2)..(2): Xaa at position 2 is α- Aminoisobutyric acid
  MOD_RES (6)..(6): Xaa at position 6 is α- Methylphenylalanine
  MOD_RES (17)..(17): Amino group of Lys side chain at position 17 is chemically modified by Fatty acid side chain groups AEEAc-AEEAc-γGlu-CO(CH2)18COOH
  MOD_RES (20)..(20): Xaa at position 20 is α- Aminoisobutyric acid
  MOD_RES (29)..(29): Xaa at position 29 is α- Aminoisobutyric acid
  MOD_RES (39)..(39): Ser at position 39 is optionally amidated
YXQGTXTSDYSIFLDKKAQXAFIEFLLEXHPSSGAPPPS

SEQ ID NO: 17 - protein, 39 aa, Artificial Sequence; identical to SEQ ID NO: 13
  MOD_RES (2)..(2): Xaa at position 2 is α- Aminoisobutyric acid
  MOD_RES (6)..(6): Xaa at position 6 is α- Methyl-2-fluorophenylalanine
  MOD_RES (17)..(17): Amino group of Lys side chain at position 17 is chemically modified by Fatty acid side chain group AEEAc-AEEAc-γGlu-CO(CH2)18COOH
  MOD_RES (20)..(20): Xaa at position 20 is α- Aminoisobutyric acid
  MOD_RES (39)..(39): Ser at position 39 is optionally amidated

SEQ ID NO: 18 - protein, 39 aa, Artificial Sequence
  MOD_RES (2)..(2): Xaa at position 2 is α- Aminoisobutyric acid
  MOD_RES (6)..(6): Xaa at position 6 is α- Methyl-2-fluorophenylalanine
  MOD_RES (17)..(17): Amino group of Lys side chain at position 17 is chemically modified by Fatty acid side chain group AEEAc-AEEAc-γGlu-CO(CH2)18COOH
  MOD_RES (20)..(20): Xaa at position 20 is α- Aminoisobutyric acid
  MOD_RES (29)..(29): Xaa at position 29 is α- Aminoisobutyric acid
  MOD_RES (39)..(39): Ser at position 39 is optionally amidated
YXQGTXTSDYSIFLDKKAQXAFIEYLLEXHPSSGAPPPS

SEQ ID NO: 19 - protein, 39 aa, Artificial Sequence; identical to SEQ ID NO: 14
  MOD_RES (2)..(2): Xaa at position 2 is α- Aminoisobutyric acid
  MOD_RES (6)..(6): Xaa at position 6 is α- Methyl-2-fluorophenylalanine
  MOD_RES (13)..(13): Xaa at position 13 is α- Methylleucine
  MOD_RES (17)..(17): Amino group of Lys side chain at position 17 is chemically modified by Fatty acid side chain group AEEAc-AEEAc-γGlu-CO(CH2)18COOH
  MOD_RES (20)..(20): Xaa at position 20 is α- Aminoisobutyric acid
  MOD_RES (39)..(39): Ser at position 39 is optionally amidated

SEQ ID NO: 20 - protein, 39 aa, Artificial Sequence
  MOD_RES (2)..(2): Xaa at position 2 is α- Aminoisobutyric acid
  MOD_RES (6)..(6): Xaa at position 6 is α- Methyl-2-fluorophenylalanine
  MOD_RES (13)..(13): Xaa at position 13 is α- Methylleucine
  MOD_RES (17)..(17): Amino group of Lys side chain at position 17 is chemically modified by Fatty acid side chain group AEEAc-AEEAc-γGlu-CO(CH2)18COOH
  MOD_RES (20)..(20): Xaa at position 20 is α- Aminoisobutyric acid
  MOD_RES (29)..(29): Xaa at position 29 is α- Aminoisobutyric acid
  MOD_RES (39)..(39): Ser at position 39 is optionally amidated
YXQGTXTSDYSIXLDKKAQXAFIEFLLEXHPSSGAPPPS

SEQ ID NO: 21 - protein, 39 aa, Artificial Sequence
  MOD_RES (2)..(2): Xaa at position 2 is α- Aminoisobutyric acid
  MOD_RES (6)..(6): Xaa at position 6 is α- Methyl-2-fluorophenylalanine
  MOD_RES (17)..(17): Amino group of Lys side chain at position 17 is chemically modified by Fatty acid side chain group AEEAc-AEEAc-γGlu-CO(CH2)18COOH
  MOD_RES (20)..(20): Xaa at position 20 is α- Aminoisobutyric acid
  MOD_RES (39)..(39): Ser at position 39 is optionally amidated
YXQGTXTSDYSIFLDKKAQXAFIEFLLEGGPSSGQPPPS

SEQ ID NO: 22 - protein, 39 aa, Artificial Sequence
  MOD_RES (2)..(2): Xaa at position 2 is α- Aminoisobutyric acid
  MOD_RES (6)..(6): Xaa at position 6 is α- Methyl-2-fluorophenylalanine
  MOD_RES (13)..(13): Xaa at position 13 is α- Methylleucine
  MOD_RES (17)..(17): Amino group of Lys side chain at position 17 is chemically modified by Fatty acid side chain group AEEAc-AEEAc-γGlu-CO(CH2)18COOH
  MOD_RES (20)..(20): Xaa at position 20 is α- Aminoisobutyric acid
  MOD_RES (39)..(39): Ser at position 39 is optionally amidated
YXQGTXTSDYSIXLDKKAQXAFIEFLLEGGPSSGQPPPS

SEQ ID NO: 23 - protein, 39 aa, Artificial Sequence; identical to SEQ ID NO: 8
  MOD_RES (2)..(2): Xaa at position 2 is α- Aminoisobutyric acid
  MOD_RES (6)..(6): Xaa at position 6 is α- Methyl-2-fluorophenylalanine
  MOD_RES (13)..(13): Xaa at position 13 is α- Methylleucine
  MOD_RES (17)..(17): Amino group of Lys side chain at position 17 is chemically modified by Fatty acid side chain group AEEAc-AEEAc-γGlu-CO(CH2)18COOH
  MOD_RES (20)..(20): Xaa at position 20 is α- Aminoisobutyric acid
  MOD_RES (39)..(39): Ser at position 39 is optionally amidated

SEQ ID NO: 24 - protein, 39 aa, Artificial Sequence
  MOD_RES (2)..(2): Xaa at position 2 is α- Aminoisobutyric acid
  MOD_RES (6)..(6): Xaa at position 6 is α- Methyl-2-fluorophenylalanine
  MOD_RES (13)..(13): Xaa at position 13 is α- Methylleucine
  MOD_RES (17)..(17): Amino group of Lys side chain at position 17 is chemically modified by Fatty acid side chain group AEEAc-AEEAc-γGlu-CO(CH2)18COOH
  MOD_RES (20)..(20): Xaa at position 20 is α- Aminoisobutyric acid
  MOD_RES (34)..(34): Xaa at position 34 is α- Aminoisobutyric acid
  MOD_RES (39)..(39): Ser at position 39 is optionally amidated
YXQGTXTSDYSIXLDKKAQXAFIEFLLETGPSSXHPPPS

SEQ ID NO: 25 - protein, 39 aa, Artificial Sequence
  MOD_RES (2)..(2): Xaa at position 2 is α- Aminoisobutyric acid
  MOD_RES (6)..(6): Xaa at position 6 is α- Methyl-2-fluorophenylalanine
  MOD_RES (13)..(13): Xaa at position 13 is α- Methylleucine
  MOD_RES (17)..(17): Amino group of Lys side chain at position 17 is chemically modified by Fatty acid side chain group AEEAc-AEEAc-γGlu-CO(CH2)18COOH
  MOD_RES (20)..(20): Xaa at position 20 is α- Aminoisobutyric acid
  MOD_RES (34)..(34): Xaa at position 34 is α- Aminoisobutyric acid
  MOD_RES (39)..(39): Ser at position 39 is optionally amidated
YXQGTXTSDYSIXLDKKAQXAFIEFLLEGRPSSXHPPPS

SEQ ID NO: 26 - protein, 39 aa, Artificial Sequence
  MOD_RES (2)..(2): Xaa at position 2 is α- Aminoisobutyric acid
  MOD_RES (6)..(6): Xaa at position 6 is α- Methylphenylalanine
  MOD_RES (13)..(13): Xaa at position 13 is α- Methylleucine
  MOD_RES (17)..(17): Amino group of Lys side chain at position 17 is chemically modified by Fatty acid side chain group AEEAc-AEEAc-γGlu-CO(CH2)18COOH
  MOD_RES (20)..(20): Xaa at position 20 is α- Aminoisobutyric acid
  MOD_RES (39)..(39): Ser at position 39 is optionally amidated
YXQGTXTSDYSIXLDKKAQXAFIEFLLESHPSSGAPPPS

SEQ ID NO: 27 - protein, 39 aa, Artificial Sequence
  MOD_RES (2)..(2): Xaa at position 2 is α- Aminoisobutyric acid
  MOD_RES (6)..(6): Xaa at position 6 is α- Methylphenylalanine
  MOD_RES (13)..(13): Xaa at position 13 is α- Methylphenylalanine
  MOD_RES (17)..(17): Amino group of Lys side chain at position 17 is chemically modified by Fatty acid side chain group AEEAc-AEEAc-γGlu-CO(CH2)18COOH
  MOD_RES (20)..(20): Xaa at position 20 is α- Aminoisobutyric acid
  MOD_RES (39)..(39): Ser at position 39 is optionally amidated
YXQGTXTSDYSIXLDKKAQXAFIEYLLESHPSSGAPPPS

SEQ ID NO: 28 - protein, 39 aa, Artificial Sequence
  MOD_RES (2)..(2): Xaa at position 2 is α- Aminoisobutyric acid
  MOD_RES (6)..(6): Xaa at position 6 is α- Methylphenylalanine
  MOD_RES (13)..(13): Xaa at position 13 is α- Methylphenylalanine
  MOD_RES (17)..(17): Amino group of Lys side chain at position 17 is chemically modified by Fatty acid side chain group AEEAc-AEEAc-γGlu-CO(CH2)18COOH
  MOD_RES (20)..(20): Xaa at position 20 is α- Aminoisobutyric acid
  MOD_RES (30)..(30): Xaa at position 30 is α- Aminoisobutyric acid
  MOD_RES (38)..(38): Xaa at position 38 is Ac3c
  MOD_RES (39)..(39): Ser at position 39 is optionally amidated
YXQGTXTSDYSIXLDKKAQXAFIEFLLESXPSSGAPPXS

SEQ ID NO: 29 - protein, 39 aa, Artificial Sequence
  MOD_RES (2)..(2): Xaa at position 2 is α- Aminoisobutyric acid
  MOD_RES (6)..(6): Xaa at position 6 is α- Methylphenylalanine
  MOD_RES (17)..(17): Amino group of Lys side chain at position 17 is chemically modified by Fatty acid side chain group AEEAc-AEEAc-γGlu-CO(CH2)18COOH
  MOD_RES (20)..(20): Xaa at position 20 is α- Aminoisobutyric acid
  MOD_RES (30)..(30): Xaa at position 30 is α- Aminoisobutyric acid
  MOD_RES (38)..(38): Xaa at position 38 is Ac3c
  MOD_RES (39)..(39): Ser at position 39 is optionally amidated
YXQGTXTSDYSIFLDKKAQXAFIEYLLESXPSSGAPPXS

SEQ ID NO: 30 - protein, 39 aa, Artificial Sequence
  MOD_RES (2)..(2): Xaa at position 2 is α- Aminoisobutyric acid
  MOD_RES (6)..(6): Xaa at position 6 is α- Methylphenylalanine
  MOD_RES (13)..(13): Xaa at position 13 is α- Methylleucine
  MOD_RES (17)..(17): Amino group of Lys side chain at position 17 is chemically modified by Fatty acid side chain group AEEAc-AEEAc-γGlu-CO(CH2)18COOH
  MOD_RES (20)..(20): Xaa at position 20 is α- Aminoisobutyric acid
  MOD_RES (30)..(30): Xaa at position 30 is α- Aminoisobutyric acid
  MOD_RES (38)..(38): Xaa at position 38 is Ac3c
  MOD_RES (39)..(39): Ser at position 39 is optionally amidated
YXQGTXTSDYSIXLDKKAQXAFIEFLLETXPSSGAPPXS

SEQ ID NO: 31 - protein, 39 aa, Artificial Sequence
  MOD_RES (2)..(2): Xaa at position 2 is α- Aminoisobutyric acid
  MOD_RES (6)..(6): Xaa at position 6 is α- Methyl-2-fluorophenylalanine
  MOD_RES (13)..(13): Xaa at position 13 is α- Methylleucine
  MOD_RES (17)..(17): Amino group of Lys side chain at position 17 is chemically modified by Fatty acid side chain group AEEAc-AEEAc-γGlu-CO(CH2)18COOH
  MOD_RES (20)..(20): Xaa at position 20 is α- Aminoisobutyric acid
  MOD_RES (29)..(29): Xaa at position 29 is α- Aminoisobutyric acid
  MOD_RES (38)..(38): Xaa at position 38 is Ac3c
  MOD_RES (39)..(39): Ser at position 39 is optionally amidated
YXQGTXTSDYSIXLDKKAQXAFIEFLLEXHPSSGAPPXS

SEQ ID NO: 32 - protein, 39 aa, Artificial Sequence
  MOD_RES (2)..(2): Xaa at position 2 is α- Aminoisobutyric acid
  MOD_RES (6)..(6): Xaa at position 6 is α- Methyl-2-fluorophenylalanine
  MOD_RES (17)..(17): Amino group of Lys side chain at position 17 is chemically modified by Fatty acid side chain group AEEAc-AEEAc-γGlu-CO(CH2)18COOH
  MOD_RES (20)..(20): Xaa at position 20 is α- Aminoisobutyric acid
  MOD_RES (29)..(29): Xaa at position 29 is α- Aminoisobutyric acid
  MOD_RES (38)..(38): Xaa at position 38 is Ac3c
  MOD_RES (39)..(39): Ser at position 39 is optionally amidated
YXQGTXTSDYSIFLDKKAQXAFIEYLLEXHPSSGAPPXS

SEQ ID NO: 33 - protein, 39 aa, Artificial Sequence
  MOD_RES (2)..(2): Xaa at position 2 is α- Aminoisobutyric acid
  MOD_RES (6)..(6): Xaa at position 6 is α- Methylphenylalanine
  MOD_RES (13)..(13): Xaa at position 13 is α- Methylleucine
  MOD_RES (17)..(17): Amino group of Lys side chain at position 17 is chemically modified by Fatty acid side chain group AEEAc-AEEAc-γGlu-CO(CH2)18COOH
  MOD_RES (20)..(20): Xaa at position 20 is α- Aminoisobutyric acid
  MOD_RES (34)..(34): Xaa at position 34 is α- Aminoisobutyric acid
  MOD_RES (38)..(38): Xaa at position 38 is Ac3c
  MOD_RES (39)..(39): Ser at position 39 is optionally amidated
YXQGTXTSDYSIXLDKKAQXAFIEFLLESHPSSXHPPXS

SEQ ID NO: 34 - protein, 39 aa, Artificial Sequence
  MOD_RES (2)..(2): Xaa at position 2 is α- Aminoisobutyric acid
  MOD_RES (6)..(6): Xaa at position 6 is α- Methyl-2-fluorophenylalanine
  MOD_RES (13)..(13): Xaa at position 13 is α- Methylleucine
  MOD_RES (17)..(17): Amino group of Lys side chain at position 17 is chemically modified by Fatty acid side chain group AEEAc-AEEAc-γGlu-CO(CH2)18COOH
  MOD_RES (20)..(20): Xaa at position 20 is α- Aminoisobutyric acid
  MOD_RES (38)..(38): Xaa at position 38 is Ac3c
  MOD_RES (39)..(39): Ser at position 39 is optionally amidated
YXQGTXTSDYSIXLDKKAQXAFIEYLLETGPSSGQPPXS

SEQ ID NO: 35 - protein, 39 aa, Artificial Sequence; identical to SEQ ID NO: 34
  MOD_RES (2)..(2): Xaa at position 2 is α- Aminoisobutyric acid
  MOD_RES (6)..(6): Xaa at position 6 is α- Methylphenylalanine
  MOD_RES (13)..(13): Xaa at position 13 is α- Methylleucine
  MOD_RES (17)..(17): Amino group of Lys side chain at position 17 is chemically modified by Fatty acid side chain groups AEEAc-AEEAc-γGlu-CO(CH2)18COOH
  MOD_RES (20)..(20): Xaa at position 20 is α- Aminoisobutyric acid
  MOD_RES (38)..(38): Xaa at position 38 is Ac3c
  MOD_RES (39)..(39): Ser at position 39 is optionally amidated

SEQ ID NO: 36 - protein, 39 aa, Artificial Sequence
  MOD_RES (2)..(2): Xaa at position 2 is α- Aminoisobutyric acid
  MOD_RES (6)..(6): Xaa at position 6 is α- Methylphenylalanine
  MOD_RES (13)..(13): Xaa at position 13 is α- Methylleucine
  MOD_RES (17)..(17): Amino group of Lys side chain at position 17 is chemically modified by Fatty acid side chain group AEEAc-AEEAc-γGlu-CO(CH2)18COOH
  MOD_RES (20)..(20): Xaa at position 20 is α- Aminoisobutyric acid
  MOD_RES (34)..(34): Xaa at position 34 is α- Aminoisobutyric acid
  MOD_RES (39)..(39): Ser at position 39 is optionally amidated
YXQGTXTSDYSIXLDKKAQXAFIEFLLEGGPSSXHPPPS

SEQ ID NO: 37 - protein, 39 aa, Artificial Sequence; identical to SEQ ID NO: 25
  MOD_RES (2)..(2): Xaa at position 2 is α- Aminoisobutyric acid
  MOD_RES (6)..(6): Xaa at position 6 is α- Methylphenylalanine
  MOD_RES (13)..(13): Xaa at position 13 is α- Methylleucine
  MOD_RES (17)..(17): Amino group of Lys side chain at position 17 is chemically modified by Fatty acid side chain group AEEAc-AEEAc-γGlu-CO(CH2)18COOH
  MOD_RES (20)..(20): Xaa at position 20 is α- Aminoisobutyric acid
  MOD_RES (34)..(34): Xaa at position 34 is α- Aminoisobutyric acid
  MOD_RES (39)..(39): Ser at position 39 is optionally amidated

SEQ ID NO: 38 - protein, 39 aa, Artificial Sequence; identical to SEQ ID NO: 24
  MOD_RES (2)..(2): Xaa at position 2 is α- Aminoisobutyric acid
  MOD_RES (6)..(6): Xaa at position 6 is α- Methyl-2-fluorophenylalanine
  MOD_RES (13)..(13): Xaa at position 13 is α- Methylleucine
  MOD_RES (17)..(17): Amino group of Lys side chain at position 17 is chemically modified by Fatty acid side chain group AEEAc-AEEAc-γGlu-CO(CH2)18COOH
  MOD_RES (20)..(20): Xaa at position 20 is α- Aminoisobutyric acid
  MOD_RES (34)..(34): Xaa at position 34 is α- Aminoisobutyric acid
  MOD_RES (39)..(39): Ser at position 39 is optionally amidated

SEQ ID NO: 39 - protein, 39 aa, Artificial Sequence
  MOD_RES (2)..(2): Xaa at position 2 is α- Aminoisobutyric acid
  MOD_RES (6)..(6): Xaa at position 6 is α- Methyl-2-fluorophenylalanine
  MOD_RES (13)..(13): Xaa at position 13 is α- Methylleucine
  MOD_RES (17)..(17): Amino group of Lys side chain at position 17 is chemically modified by Fatty acid side chain group AEEAc-AEEAc-γGlu-CO(CH2)18COOH
  MOD_RES (20)..(20): Xaa at position 20 is α- Aminoisobutyric acid
  MOD_RES (34)..(34): Xaa at position 34 is α- Aminoisobutyric acid
  MOD_RES (39)..(39): Ser at position 39 is optionally amidated
YXQGTXTSDYSIXLDKKAQXAFIEFLLETRPSSXHPPPS

SEQ ID NO: 40 - protein, 39 aa, Artificial Sequence; identical to SEQ ID NO: 33
  MOD_RES (2)..(2): Xaa at position 2 is α- Aminoisobutyric acid
  MOD_RES (6)..(6): Xaa at position 6 is α- Methyl-2-fluorophenylalanine
  MOD_RES (13)..(13): Xaa at position 13 is α- Methylleucine
  MOD_RES (17)..(17): Amino group of Lys side chain at position 17 is chemically modified by Fatty acid side chain group AEEAc-AEEAc-γGlu-CO(CH2)18COOH
  MOD_RES (20)..(20): Xaa at position 20 is α- Aminoisobutyric acid
  MOD_RES (34)..(34): Xaa at position 34 is α- Aminoisobutyric acid
  MOD_RES (38)..(38): Xaa at position 38 is Ac3c
  MOD_RES (39)..(39): Ser at position 39 is optionally amidated

SEQ ID NO: 41 - protein, 39 aa, Artificial Sequence
  MOD_RES (2)..(2): Xaa at position 2 is α- Aminoisobutyric acid
  MOD_RES (6)..(6): Xaa at position 6 is α- Methyl-2-fluorophenylalanine
  MOD_RES (17)..(17): Amino group of Lys side chain at position 17 is chemically modified by Fatty acid side chain group AEEAc-AEEAc-γGlu-CO(CH2)18COOH
  MOD_RES (20)..(20): Xaa at position 20 is α- Aminoisobutyric acid
  MOD_RES (34)..(34): Xaa at position 34 is α- Aminoisobutyric acid
  MOD_RES (38)..(38): Xaa at position 38 is Ac3c
  MOD_RES (39)..(39): Ser at position 39 is optionally amidated
YXQGTXTSDYSILLDKKAQXAFIEFLLESHPSSXHPPXS

SEQ ID NO: 42 - protein, 39 aa, Artificial Sequence; identical to SEQ ID NO: 41
  MOD_RES (2)..(2): Xaa at position 2 is α- Aminoisobutyric acid
  MOD_RES (6)..(6): Xaa at position 6 is α- Methylphenylalanine
  MOD_RES (17)..(17): Amino group of Lys side chain at position 17 is chemically modified by Fatty acid side chain group AEEAc-AEEAc-γGlu-CO(CH2)18COOH
  MOD_RES (20)..(20): Xaa at position 20 is α- Aminoisobutyric acid
  MOD_RES (34)..(34): Xaa at position 34 is α- Aminoisobutyric acid
  MOD_RES (38)..(38): Xaa at position 38 is Ac3c
  MOD_RES (39)..(39): Ser at position 39 is optionally amidated

SEQ ID NO: 43 - protein, 39 aa, Artificial Sequence
  MOD_RES (2)..(2): Xaa at position 2 is α- Aminoisobutyric acid
  MOD_RES (6)..(6): Xaa at position 6 is α- Methyl-2-fluorophenylalanine
  MOD_RES (13)..(13): Xaa at position 13 is α- Methylleucine
  MOD_RES (17)..(17): Amino group of Lys side chain at position 17 is chemically modified by Fatty acid side chain group AEEAc-AEEAc-γGlu-CO(CH2)18COOH
  MOD_RES (20)..(20): Xaa at position 20 is α- Aminoisobutyric acid
  MOD_RES (34)..(34): Xaa at position 34 is α- Aminoisobutyric acid
  MOD_RES (38)..(38): Xaa at position 38 is Ac3c
  MOD_RES (39)..(39): Ser at position 39 is optionally amidated
YXQGTXTSDYSIXLDKKAQXAFIEYLLESHPSSXHPPXS

SEQ ID NO: 44 - protein, 39 aa, Artificial Sequence
  MOD_RES (2)..(2): Xaa at position 2 is α- Aminoisobutyric acid
  MOD_RES (13)..(13): Xaa at position 13 is α- Methylleucine
  MOD_RES (17)..(17): Amino group of Lys side chain at position 17 is chemically modified by Fatty acid side chain group AEEAc-AEEAc-γGlu-CO(CH2)18COOH
  MOD_RES (20)..(20): Xaa at position 20 is α- Aminoisobutyric acid
  MOD_RES (39)..(39): Ser at position 39 is optionally amidated
YXQGTFTSDYSIXLDKKAQXAFIEYLLEGGPSSGAPPPS

SEQ ID NO: 45 - protein, 39 aa, Artificial Sequence
  MOD_RES (2)..(2): Xaa at position 2 is α- Aminoisobutyric acid
  MOD_RES (13)..(13): Xaa at position 13 is α- Methylleucine
  MOD_RES (17)..(17): Amino group of Lys side chain at position 17 is chemically modified by Fatty acid side chain group AEEAc-AEEAc-γGlu-CO(CH2)18COOH
  MOD_RES (20)..(20): Xaa at position 20 is α- Aminoisobutyric acid
  MOD_RES (29)..(29): Xaa at position 29 is α- Aminoisobutyric acid
  MOD_RES (39)..(39): Ser at position 39 is optionally amidated
YXQGTFTSDYSIXLDKKAQXAFIEYLLEXGPSSGAPPPS